European Patent Application EP 4 715 056 A1, published March 25, 2026. Title: 一种生物基反式乌头酸酯及其制备方法和应用. Applicant: 中国科学院青岛生物能源与过程研究所. The sequence listing filed with the application follows.

SEQUENCE LISTING (139 sequences)

SEQ ID NO: 1 - protein, 357 aa, synthetic construct
MKIPCFVMRGGTSKGLFFLDKHLPSNKSIRDEVILKALGAGNARGVDGMGTLDPLSNKIAIIRISTTPGIDIDYLFLQADLKRRILDDSVNCGNIIAAVAPYAVESGLIKVGSGKETITIRNLNTNVIVESTIATKNGNVVYNGDIKIDGVPGTGAPIDLNFKNSIGSVTGKLFPTGAKTDVINGINVSCVDVSVPLIIIRASELGIIGNESPDVLNANKTFLHDIDLIRKKVACLANLGDVSNKVIPKIAVISKPRESGTITSRYFIPHQCHSTHAVTGSLALSAAIKINGTTAYHVAKNNDLNKMKKLNQIIIEHPAGKIQTESVIEESSNGYVIKKSSITRTARLLFKGELIIP

SEQ ID NO: 2 - protein, 443 aa, synthetic construct
MLHPIDTTIYRAGTSRGLYFLASDLPAEPSERDAALISIMGSGHPLQIDGMGGGNSLTSKVAIVSASTQRSEFDVDYLFCQVGITERFVDTAPNCGNLMSGVAAFAIERGLVQPHPSDTTCLVRIFNLNSRQASELVIPVYNGRVHYDDIDDMHMQRPSARVGLRFLDTVGSCTGKLLPTGNASDWIDGLKVSIIDSAVPVVFIRQHDVGITGSEAPATLNANTALLDRLERVRLEAGRRMGLGDVSGSVVPKLSLIGPGTETTTFTARYFTPKACHNAHAVTGAICTAGAAYIDGSVVCEILSSRASACSASQRRISIEHPSGVLEVGLVPPENAAQSLVDVAVVERSIALIAHARVYYTTPDRRRSYDSPLTSPSTPADTHNLFDAAYRPVIQPSDTDVEAPHMLALENKEQCVSRCDTALHHIVASYGASDAHASDRSLS

SEQ ID NO: 3 - DNA, 1074 bp, synthetic construct
  source 1..1074: mol_type = other DNA
atgaagatcccctgcttcgtcatgcgcggcggcaccagcaagggcctgttcttcctggacaagcacctgccctccaacaagtccatccgcgacgaggtcatcctgaaggccctgggcgccggcaacgcccgtggtgtcgatggtatgggcaccctggaccccctgagcaacaagatcgccatcatccgcatcagcaccacccccggcatcgacatcgactacctgttcctgcaagccgacctgaagcgccgcatcctggacgacagcgtcaactgcggcaacatcatcgccgccgtcgccccctacgccgtcgaatctggcctgatcaaggtcggcagcggcaaggagaccatcaccatccgcaacctgaacaccaacgtcatcgtcgagagcaccatcgccaccaagaacggcaacgtcgtctacaacggcgacatcaagatcgacggcgtccccggcaccggcgctcctattgacctgaacttcaagaacagcatcggcagcgtcaccggcaagctgttccccaccggcgccaagaccgacgtcatcaacggcatcaacgtctcctgcgtcgacgtcagcgtccccctgatcatcatccgcgcctccgagctgggcatcatcggcaacgagagccccgacgtcctgaacgccaacaagaccttcctgcacgacatcgacctgatccgcaagaaggtcgcctgcctggccaacctgggcgacgtctccaacaaggtcatccccaagatcgccgtcatcagcaagccccgcgagtccggcaccatcacctcccgttacttcatcccccaccagtgccactccacccacgccgtcaccggcagcctggctctgtccgctgccatcaagatcaacggcaccaccgcctaccacgtcgccaagaacaacgacctgaacaagatgaagaagctgaaccagatcatcatcgagcaccccgccggcaagatccagaccgagtccgtcatcgaggagtcctccaacggctacgtcatcaagaagagctccatcacccgcaccgcccgcctgctgttcaagggcgagctgatcatcccctaa

SEQ ID NO: 4 - DNA, 1332 bp, synthetic construct
  source 1..1332: mol_type = other DNA
atgctgcaccccatcgacaccaccatctaccgcgccggcaccagccgcggtctgtacttcctggcctccgacctgcccgccgagccttctgagcgcgacgctgctctgatctccatcatgggctccggccaccccctgcaaatcgacggcatgggcggcggcaactccctgacctccaaggtcgccatcgtctccgcctccacccagcgcagcgagttcgacgtcgactacctgttctgccaggtcggcatcaccgagcgcttcgtcgacaccgcccccaactgcggcaacctgatgtccggcgtcgccgccttcgccatcgagcgtggtctggtccagccccacccctccgacaccacctgcctggtccgcatcttcaacctgaactcccgccaggcctccgagctggtcatccccgtctacaacggccgcgtccactacgacgacatcgacgacatgcacatgcagcgccccagcgcccgcgtcggtttgcgtttcctggacaccgtcggcagctgcaccggcaagctgctgcccaccggcaacgccagcgactggatcgacggcctgaaggtcagcatcatcgactccgccgtccccgtcgtcttcatccgccagcacgacgtcggcatcacgggcagcgaggcccctgctaccctgaacgccaacaccgccctgctggaccgcctggagcgcgttcgtctggaggccggtcgccgtatgggcctgggtgacgtctccggcagcgtcgtccccaagctgagcctgatcggccccggcaccgagaccaccaccttcaccgcccgctacttcacccccaaggcctgccacaacgcccacgccgtcaccggtgccatctgcaccgccggtgccgcttacatcgacggcagcgtcgtgtgcgagatcctgtccagccgcgcctccgcctgctccgcttctcagcgtcgcatcagcatcgagcaccccagcggcgtcctggaggtcggtctggtcccccctgagaacgccgcccagtccctggtcgacgtcgccgttgtcgagcgcagcatcgccctgatcgcccacgcccgtgtctactacaccacccccgaccgccgccgctcctacgatagccctctgacctccccctccacccccgctgacacccacaacctgttcgacgccgcctaccgccccgtcatccagcctagcgacaccgacgtcgaggccccccacatgctggccctggagaacaaggagcagtgcgtctcccgctgcgacaccgccctgcaccacatcgtcgcctcctacggcgccagcgacgcccatgctagcgaccgtagcctgtcctaa

SEQ ID NO: 5 - protein, 786 aa, synthetic construct
MISTRLARMGALAPKSRLLLGTRGLATVADSPLDKKVEMTNHEKGNYINYKKMSENLDIVRRRLSRPLTYAEKVLYSHLDDPHGQDIERGVSYLKLRPDRVACQDATAQMAILQFMSAGMPSVATPTTVHCDHLIEAQVGGEKDLARANEINKEVYDFLATATAKYNIGFWKPGSGIIHQIVLENYAFPGGLMIGTDSHTPNAGGLAMAAIGVGGADAVDVMAGLPWELKAPKVIGVKLTGEMSGWTTPKDIILKVAGLLTVKGGTGAIIEYHGPGVNSLSCTGMGTICNMGAEIGATTSMFPFNDRMYDYLKATKRQHIGEFARSYAKELREDEGAEYDQLIEINLSELEPHINGPFTPDLATPISKFKEAVDANGWPEELKVGLIGSCTNSSYEDMSRAASIARDALNHGVKSKSLFTVTPGSEQIRATIERDGQLQTLEEFGGVILANACGPCIGQWDRKDVKKGEPNSIISSYNRNFTGRNDANPATHAFVASPDLVVAMCVAGTLKFNPLTDTVKDKDGKEFKLAPPSGDGLPSKGYDAGRNTYQAPPQDRASINVAVSPTSDRLQLLAGFEAWDGKDANGIPILIKCQGKTTTDHISMAGPWLKYRGHLDNISNNMLIGAVNAENGEANKVKNKFTGEYGAVPATARDYKARGVKWVVIGDWNYGEGSSREHAALEPRHLGGLAIITRSFARIHETNLKKQGMLPLTFADPADYDKIQPEDTVDLLCTELEVGKPMTLRVHPKNGSTFDVKLNHTFNESQIEWFKDGSALNTMARKAASN

SEQ ID NO: 6 - DNA, 2837 bp, synthetic construct
  source 1..2837: mol_type = other DNA
atgatctccacccgccttgcgcgcatgggtgcgctggtaagtcttctctcccagatcgcgaccgtggtatctcgccagaaacaagataccagctgtcgcaaactcgacctagaaatcgaccgaaagctaatccctttctccgacaggcccccaagtcccgtcttgtaagcttttccccgcgaccgtcagatactccttgcgagactctgggagagacgagatcggaacctcaggattctttggaaacatggatactaactatctcgatagcttctcgggacccggggtctggccaccgttgctgattcccctctggacaagaaggtcgagatgaccaaccacgagaaggtgagtggtttctaccgagttcggctatcttcggatggcgaatgtcaccctgtttgggaagacaccattggctaattctgcatacagggtaactacatcaactacaagtatgccaattccttgcgcaaacctgatgggaccatttgcacgatcatgggaaaacccggattggatggcccgagggtcaaatcggctgtgcgctaacatgtgctccacctttgtaggaagatgtccgagaacctggacattgtccgtcgccgtctgagccgccctctcacctacgccgagaaggttctctattctcaccttgatgatcctcatggtcaggacatcgagcgtggtgtttcttacctgaagctccgccccgaccgtgtcgcttgccaggatgctactgctcagatggctatcctgcagttcatgtccgctggcatgccttccgtcgctacccccaccaccgtgcactgcgaccacttgattgaggctcaggttggtggtgagaaggatcttgctcgtgccaacgagatcaacaaggaggtctacgacttcctggccaccgccaccgccaagtacaacatcggtttctggaagcccggttccggtatcattcaccagatcgtcctggagaactatgcgttccccggtggtctgatgatcggtactgactctcacactcctaacgctggtggtcttgctatggctgccattggtgtcggtggtgctgatgccgtcgatgtcatggctggtctcccttgggagttgaaggcccccaaggtcattggtgtcaagctgactggtgagatgtccggatggaccactcctaagggtaagttgcaaaatttgcgcatccgatcggccttgcaatcgctgacagcgccatagatatcatcctgaaggtcgctggtctcctgactgtcaagggtggtactggtgccatcattgagtaccacggtcctggtgtcaactccctgtcttgcactggtatgggtaccatctgtaacatgggtgctgaaattggtgctaccacctccatgttccccttcaacgaccgcatgtacgactacctgaaggccaccaagcgtcagcacattggtgagttcgcccgctcctacgccaaggagctccgcgaggatgagggtgccgagtacgaccagctcattgagatcaacctctctgagcttgagccccacatcaacggtcccttcacccccgacttggccacccccatctccaagttcaaggaggctgttgatgccaacgggtggcccgaggagctcaaggtcggtctgatcggctcttgcaccaactcctcttacgaggatatgtcccgtgcggcctccatcgcccgtgacgccctcaaccacggcgtgaagtccaagtctctcttcactgtcacccccggttctgagcagatccgcgccaccattgagcgtgacggccagctccagaccctcgaggagttcggcggtgtcatccttgccaacgcctgcggtccttgcatcggtcagtgggatcgtaaggacgtgaagaagggtgagcccaactccatcatctcttcttacaaccgtaacttcaccggtcgtaacgatgccaaccctgccactcacgctttcgtcgcctcccctgaccttgtcgttgccatgtgtgttgctggcaccctcaagttcaaccctctcaccgatactgtgaaggacaaggatggcaaggagttcaagcttgctcctccttctggtgatggtctccccagcaagggctacgacgccggccgcaacacctaccaggctcctcctcaggaccgtgcgtccatcaacgtcgctgtctcccccactagcgaccgtctccagctcctcgctggctttgaggcctgggatggcaaggatgccaacggcattcccatcctgatcaagtgccagggcaagaccaccactgaccatatctccatggctggcccatggttgaagtaccgtggccacttggacaacatctccaacaacatgcttatcggtgccgttaacgctgagaacggcgaggccaacaaggtcaagaacaagttcaccggcgaatacggtgccgtccccgctaccgctcgtgactacaaggcccgtggtgtgaagtgggttgtcattggtgactggaactacggtgagggctcttctcgtgagcacgctgctcttgagccccgtcaccttggtggtctggccatcatcacccgttctttcgcccgtatccacgagaccaacctgaagaagcagggtatgcttcctctgaccttcgctgaccccgccgactacgacaagatccagcctgaggacaccgtcgacctcctctgcaccgagcttgaggtcggcaagcccatgaccctccgtgtccaccccaagaatggctctaccttcgacgtcaagctcaaccacacctttaacgagtcccagatcgagtggttcaaggacggatccgcccttaacaccatggcccgcaaggctgctagcaactaa

SEQ ID NO: 7 - protein, 32 aa, synthetic construct
MISTRLARMGALAPKSRLLLGTRGLATVADSP

SEQ ID NO: 8 - protein, 34 aa, synthetic construct
MAASLRLGTSALRSTTLAGKPVVQSAAFNGLRCY

SEQ ID NO: 9 - protein, 84 aa, synthetic construct
MSSVRFSSALARRSFAVASPPLSAPLSSSARRFLSSSSSISSSSSSVSTRSPRSLTSASSLLSSRTASARWTGLSSLNLTQSRT

SEQ ID NO: 10 - DNA, 1984 bp, synthetic construct
  source 1..1984: mol_type = other DNA
ggattgcctgaacattgacattcggcgtccggccgggaccaccgcggactcgaagctgcctgtgctggtctggatctttggcggaggctttgaacttggttcaaaggcgatgtatgatggtacaacgatggtatcatcgtcgatagacaagaacatgcctatcgtgtttgtagcaatgaattatcgcgtgggaggtttcgggttcttgcccggaaaggagatcctggaggacgggtccgcgaacctagggctcctggaccaacgccttgccctgcagtgggttgccgacaacatcgaggcctttggtggagacccggacaaggtgacgatttggggagaatcagcaggagccatttccgtttttgatcagatgatcttgtacgacggaaacatcacttacaaggataagcccttgttccggggggccatcatggactccggtagtgttgttcccgcagaccccgtcgatggggtcaagggacagcaagtatatgatgcggtagtggaatctgcaggctgttcctcttctaacgacaccctagcttgtctgcgtgaactagactacaccgacttcctcaatgcggcaaactccgtgccaggcattttaagctaccattctgtggcgttatcatatgtgcctcgaccggacgggacggcgttgtcggcatcaccggacgttttgggcaaagcagggaaatatgctcgggtcccgttcatcgtgggcgaccaagaggatgaggggaccttattcgccttgtttcagtccaacattacgacgatcgacgaggtggtcgactacctggcctcatacttcttctatgacgctagccgagagcagcttgaagaactagtggccctgtacccagacaccaccacgtacgggtctccgttcaggacaggcgcggccaacaactggtatccgcaatttaagcgattggccgccattctcggcgacttggtcttcaccattacccggcgggcattcctctcgtatgcagaggaaatctcccctgatcttccgaactggtcgtacctggcgacctatgactatggcaccccagttctggggaccttccacggaagtgacctgctgcaggtgttctatgggatcaagccaaactatgcagctagttctagccacacgtactatctgagctttgtgtatacgctggatccgaactccaaccggggggagtacattgagtggccgcagtggaaggaatcgcggcagttgatgaatttcggagcgaacgacgccagtctccttacggatgatttccgcaacgggacatatgagttcatcctgcagaataccgcggcgttccacatctgatgccattggcggaggggtccggacggtcaggaacttagccttatgagatgaatgatggacgtgtctggcctcggaaaaggatatatggggatcataatagtactagccatattaatgaagggcatataccacgcgttggacctgcgttatagcttcccgttagttatagtaccatcgttataccagccaatcaagtcaccacgcacgaccggggacggcgaatccccgggaattgaaagaaattgcatcccaggccagtgaggccagcgattggccacctctccaaggcacagggccattctgcagcgctggtggattcatcgcaatttcccccggcccggcccgacaccgctataggctggttctcccacaccatcggagattcgtcgcctaatgtctcgtccgttcacaagctgaagagcttgaagtggcgagatgtctctgcaggaattcaagctagatgctaagcgatattgcatggcaatatgtgttgatgcatgtgcttcttccttcagcttcccctcgtgcagatgaggtttggctataaattgaagtggttggtcggggttccgtgaggggctgaagtgcttcctcccttttagacgcaactgagagcctgagcttcatccccagcatcattacacctcagca

SEQ ID NO: 11 - DNA, 745 bp, synthetic construct
  source 1..745: mol_type = other DNA
ttacactctgggaggatccaggtacttccattcttactaggaagtatttcggcctagactaatacaacgaaagaaactgttcgattctacgggaaaagtactccaattccattacatcatcgcattctccctctcgtaaggtacctaccacaaacccccactatcgttcatccgtccccggttacaacgggaagaaaaagcccggggagagggggaagaagaaaatcccaagggacgggaatagccgtgcggaagagaagacgattagcctaggtagaagcctcatggccgaccatttgattccgaaaagctggcaaaacattcacgagatagacacagtgaggacccggacgatgccctatgcggcgcgctgattggccaggccgggcagtgccgaagcagcaaatatcgtgagtctcctgctttgcccggtgtatgaaaccggaaagggttgctggggagctggtcagcggcgcaagccgggagggcgactgagctctgtagcttttgccccgtctgtccgtccggtgtagagtggcagaccaccgcctgctgcgcctcccattgggtcttccccaacgtgactgggtcgttgcgtcagtccatgtcgctgcctttttcttcctccccctcccccgctgtccttcttcttcttcttcttctctctttctcccatcatcctctcatcctctgcctttcccatcgaactcacttcttctaccaacaactcatcaatcatcacaac

SEQ ID NO: 12 - DNA, 1200 bp, synthetic construct
  source 1..1200: mol_type = other DNA
ttgatcgagacctaatacagcccctacaacgaccatcaaagtcgtatagctaccagtgaggaagtggactcaaatcgacttcagcaacatctcctggataaactttaagcctaaactatacagaataagatggtggagagcttataccgagctcccaaatctgtccagatcatggttgaccggtgcctggatcttcctatagaatcatccttattcgttgacctagctgattctggagtgacccagagggtcatgacttgagcctaaaatccgccgcctccaccatttgtagaaaaatgtgacgaactcgtgagctctgtacagtgaccggtgactctttctggcatgcggagagacggacggacgcagagagaagggctgagtaataagcgccactgcgccagacagctctggcggctctgaggtgcagtggatgattattaatccgggaccggccgcccctccgccccgaagtggaaaggctggtgtgcccctcgttgaccaagaatctattgcatcatcggagaatatggagcttcatcgaatcaccggcagtaagcgaaggagaatgtgaagccaggggtgtatagccgtcggcgaaatagcatgccattaacctaggtacagaagtccaattgcttccgatctggtaaaagattcacgagatagtaccttctccgaagtaggtagagcgagtacccggcgcgtaagctccctaattggcccatccggcatctgtagggcgtccaaatatcgtgcctctcctgctttgcccggtgtatgaaaccggaaaggccgctcaggagctggccagcggcgcagaccgggaacacaagctggcagtcgacccatccggtgctctgcactcgacctgctgaggtccctcagtccctggtaggcagctttgccccgtctgtccgcccggtgtgtcggcggggttgacaaggtcgttgcgtcagtccaacatttgttgccatattttcctgctctccccaccagctgctcttttcttttctctttcttttcccatcttcagtatattcatcttcccatccaagaacctttatttcccctaagtaagtactttgctacatccatactccatccttcccatcccttattcctttgaacctttcagttcgagctttcccacttcatcgcagcttgactaacagctaccccgcttgagcagacatcacc

SEQ ID NO: 13 - DNA, 1000 bp, synthetic construct
  source 1..1000: mol_type = other DNA
tggcaccggtccgcgggatgactctcggtaggcctcggctcaggttcggctcagtctgccaggccattttccatgccggccgtaatttatgacgtttccattgcttcggcacgacgactccgggaaggcatcgtccactggggtttcaggtgaaataatcctctgaatgggccagagaaatgacctccgatgtgtgtctaaggctctatagtagaagccgcggatatttgtcggccttgatcctcccaattaattatatccactccagaccactaatagtatatcggagtgtacacagttcctatgagagtaagtacctcaaactcggagaaaggtggaatgtatgatgtaagtgaggagccgaaagtaggtgtaatccttcatctctgattggaggagccacgttgtctgctcacatgcgacctccgtcgttgcggtattcgtatggtaattacagacgtattgacgatgcggacatgggggtatggggtatgtgggtaggtaaataatcagttcgttatagggagagatctagggctacaagaaccagccatggggagaaagtctcgaatttcttcagcatccgtgaatacttaaacaccgcagattatccttttcctagaagaaataactcatagatcaaaaaaggggctggaaaacaccctcaaacacggagacaggagcggaaagtgggcaggagttactaggtccatccatgtctccggctgaatgcgtcggtattgtcacgagcggttacggttcttcttcgccggttcagaatacccaaattctttcccactctgaaaaacaaccaagcttccttttaatcgtctccatctctccgtaaacccttttctcttctctctcctctctctctccctctccactccatccttttttcttcgctacttccaatcacttgaagttagcttcttgcttggattagctctctctttgtatgtgttgcggctgtgtccacctcgcatagagagcttccatc

SEQ ID NO: 14 - DNA, 609 bp, synthetic construct
  source 1..609: mol_type = other DNA
caaccaaggaccgcgatgaccgcattctgaatgcgggatatggaagagggagggatcaattcaattccaatatataacataggtataatagatagggctgaattataagatagaatatcataaagaaaagaaaagaaaaaaaggaaaaagaaaaacctttcacaggattgaaaaccctggataaattgcaaaaaaaaataaaaaaataaaaaggtaggacaaattaattacttgttccgcgaaacggaatttggcgggtacggggacaaacacaacccaaaacatgtccaagctgccgattttctctcggtagcccggacagcccgggggccacgggcctgccgttaccatactgtaccgatttccgccattgccagcccgccttgccgatcgttaccgtacagtccgcgtaccggctgtatggtgacggtcagatggagaaaaaaaaaagaaaaaaagcgaccgcaaaagagcttctcccgcgatttgatccttcctctcttctcttccctttcccccctttgttgtgtccttgttataccctcctctcctctcttccatccttcccttcaaacagtctatcttttttagactcttgttggattcaaa

SEQ ID NO: 15 - DNA, 925 bp, synthetic construct
  source 1..925: mol_type = other DNA
ctttaacgttgcagatacagggatgcgaacagattcgcagaaaagcaaattacgtgggatgtggtccggtgcatttggggtgtgaccattaaagttgcgagttacggcatatactgaggggaggtatacgtacctgcattgcggagggactcatcttatcttgatcaagattgatggcggcggacattgagcaggggagggaggaatggagagagtctggagtactccgtaggcgggaacggaatagcgcagcattggttgtaaggaagagggtctgatgccaccacggactgcaggttgaccggacccagttctcaatggaaaaaaagtagtgtaacttccaagggaagggaacttttccccccagtctgagtctgagagtcgaatagtccggcttcggcgaccagaaagtcacaacggtgggcggaaaaggaagtgggtgtgtgtcaactccaagccttgggagggaacaaccacgccggataagaggtgttggggaccctccatttgcctttcctccctctctctctctcctctccgttcttccctcttcctccaccaaggtctcgatttgtctctgcgtctctttgcttattgcaggaagattatttccctgagcgaacagaacgattttccgggttctccgatctgccccgtgaaggtcccttaaaccagcagcatctcgtccagtccggcttaacggcagcttccgaactccaccaccgcctccttccagccgagagcttcacggcttgttgcttgtctttccctcgggtactctctctccctccccttctcgttgcccccaagtttccccttgcagcgtggattgcgatcctcctcgtttccccgtacccgataaactgatccgcttgggcagactttcccccggttcctcccacgcaggccacgcttcactgtcgaa

SEQ ID NO: 16 - DNA, 2048 bp, synthetic construct
  source 1..2048: mol_type = other DNA
ctaccaacagtctcgcggtgaatagaaaactgaccttcaaattccagcacggcgaacgaacagcatccatttttcagtttgggcgcgtcaagaacttgtagaccttctcgtagctggccgctctgtcagtcaagaataccatgtctttagattactcctcaacttacacgggaaacatgatggccgaggtaagggaaagtctccctgtccgaaaccagacaccggaccagaacacgccaatgccttcactgcgcaggagcgtcttcacgcagttgaaggtatttccgtacaattgcctagcctgaagagattgcattctggtaaacccaagtcggatccaaatcagcatatacttatctgggcggttcactatctgtctgaccagcacttaccgcgtcttgatcacgtccagtggctgtgtcgaccaggcgcagcaaactccagtaacagaaccgaccaaggtgcttgccagagggtgcacgtcttcgccattatgtgagtattttcgggccagcccaataagttcgttataaacagtgaacttcactgccgcattggacgactgccgcaaaattgtaggaccaaccgcagagaagaatccaagtggtccccgatctcgaaggattccggctatcgcgccgaaagtcgtacttaactctgcatttccaaccttccttgcatcaatgctaagagaacgaattaagaactggtcggataacgggtgagatgttgcaacttacattttcgtcttgatcgcctccgctggggttacggctaagacagcctcggtcacgccagccccaaacccagccagcatggaagctccagttgaaatttctccatttgggcccgcaagggccgagcgataaatgttgaacgaggcaaattctgtttgttattgcaaacggtcatttcttttcgttccacgcgggcttataagtggatcgctacatacgaacggaggctttcatgtggttcctaccaaggtggctccatatccagcataccagcctcggattccaggtcttatagctgccacatcatggtttcgccgcttaagctgggcgcgagttttagccgctaccagccgaagcaatagactgtcagttggcggccacggtaagcagaattcttaaacacaagatatgctcacattcgaaagggtaggtgatggagatttcaacagccccagcacaagcacccgcaaccaatgcaggaatacctttcgtctatacatatattaagaaaagacattgtcagtatcatggcccaagcgcgaccaagaaggaacacatacacgcttgccacgagctttttgggtaaggggtgcctttggtaatggaacacttgtctggactttagagtccatgacggcgatgtgctgagtccaaacaaagcttttcttcacagagatagggctgtagactttatttccagtttgccttccctgtgttcagtatcgggtcttatattgtattatctcaatgcttatgactctgagtggaatgcattggatatcagtttgtcacggagtcggcacccgatggctatcgcaatcgtccctggtgggtcttgaaatcgtatgccacacttgctccggatgaaacacattccggagcgcgcatcgatattgctacacagtatagacccaatggtctgcagatgccctaaatggtagttctcactggcctgcattaagttctggttgcagatcattgtcggcctaacatcagtgtaggttacggtgtgagatttacttgcatagaagattccagaccacaaggttctagatcctttgacggcggactcccctcgaggtgccgggcgccgacgtgtgcgttgctccgggatttgtaggacgcagctcggatacctagccgttatgggaatcggaggttgtagcagcgtaaacacatggatagttaaataatcggatgtacacccactgttggaaatgacgggggcctaacaacacgagattatctgatccaatttctgttcgttggcattctatcattcgcagcgaaaattgtcctattaaattgacc

SEQ ID NO: 17 - DNA, 1502 bp, synthetic construct
  source 1..1502: mol_type = other DNA
gtacagtggccatgaaatccaatcatttccttctggccgccctcgggcaagagatagtgccgcagaggtctctcacagcatctacatctgcgaccgcaacagccaccaagcgaggcgcacatgagcttgtcctcctcccatgccaaagtttggccctcttcgtttctgtgatgctgaaggaagtcaaactcgtcgatgataggaccagatggtttgtcaagggtcaacgctttccatgccttctggcaccggtagtaatgctcttctgcaagggagacttgacgtttcggatccgcgggccccgggacatgctggaagggattttctggctcaataccacgtctgtatttgaccctttccagacagttaatccgctgcaggagggcgaactgtagctcctcgttctccttgtagcgcttgatccagtctttttggatgttgcacttgcttggcctatgcttctcatataatcttgccctgtcatagagacgacgtctgagattgtagcgttcgtctttgatcacccggagccagataggcctgagtatatctgacattagatcaaagggtctgtggatagtctccttcagcatcagcgacgcatgtgactcgcatgtcggagagagcttgtgggtggtcatctttgatggcgtcctctgctttcccttgattttcgttgattgtttttcgaaagttaagtctggaagtcaagagaatccttctgccagacattatatttacgtatactgacgtagtagaaacagcgtcaggatgaggacatggtgtgtgctggaccacggaatcatagttcatcagtatattgggttggacaaataacgctgagcatgtatatgtctttacacactataaaagccagcgaacgccaataaaatagggcatattgatgtgaaaatatgacaccagttaaaagcagtgtattgattttatctctcttcacctcggacctatactaccgtatacaagactcaacttacttccagatatagtaatatacaccctatggacgaaccagcacaataattacagccaaacaacaccacccaaatggcatattcctaatcagcactaagcacaaataccactgtcatcacagcataatcaataagaatcccagacaaccgactcactctgactcaccttacacaaacccccaagcaaagcgcagcccagaacctcagccaacaatcgggcaacgtacggggaaagattggccgatccatgatgtcagcagccctaacccaaagcggactagcgcataccgcccctctgactccgccatcccagggctcgagaagcttccgtggcgtcgatataaattcagcgggccttgaacatccctccttacgacacacctcacgcgatcgattttgacactcacacaccgccaccctcacatcctccacccacaccacaccccttaatcaacccaccatcaccgctagaacgtctatctcatcaccgacttctcatccatcttcaaa

SEQ ID NO: 18 - DNA, 1489 bp, synthetic construct
  source 1..1489: mol_type = other DNA
ctgctctctctctgctctctttctgcgctctctgtgtcggcactaaccccgaatggggcgggtatcggcagtccgacggatctccgggggccgcacgtccagcgccgatcgttactcaaccgagcagaggagagagagcagtgagcagtggtgtcaccgaccataaaaatgcttgcttctgcccatccagccatcagttgtccagtctgctccattgtgtgccagtctcgcccccaaggccgcgcatctgaaaccaaccggttgggtgaaatcagccggcgggtggcacccgagcggccactggctgggatcatcgcccgcaacgcgtcaacagcaatcaaacgaaggatgcgaaattattcagcgggcggttcctttccatttttcccgttcctgtcagcatctctactctatcatactgtaacattattatattgtgattatttttattctgggtgatgtgtccactggaccgcacgtggaatgaagattttccttccctcgggacgagaaaccatggcgcagttggtgttgtgtgcgtgtgtgtgcgtgtcggctgtccgaaaatcgccctaaactccgaggcacgcaccatttgccattaattcccttgcgattgatttctgcctgtccctgcgaccctttgtgaccctttgtgaccctttgaccctggattcaggggcttggtggactcatagcgatggggatagggacttttgacccttttgaccctttgaccctcccattttccctggcctaagtacgctgtagtcgtaattatagaaagaatcttgcgtggactggggcaaaaggggaacagaacttatccatgtccgagcagcgatcggccagtcaccaagccggctggatccgagacccgctacgtgggaactcccaagagtcgttaagcaaagccaagagatcagccaagatgtcgctcacgagcctaattgctggattgccatatcgcttgtcgttgtaccatcgcgtaagattttatcattgtttctgggggctgtcagctagtctaaaacgtactcctcaaaccagagaggctgatgatgctgatgatgggcctccacccccccaaattggtagcgccgttccatgagaggcccagtctctctgcccgtcctcgaccattgtttggcccagcactgacacaaccttcagggggggccaatggacgtattccgtaggcagcaggcaaatgcggccctaagaactccccaactaataagagtccagactagcaaaggttcgcctcgccggtctccatctcttccttcttagtcctcccatttcctccctcccacttggtctctcgctccagatttcctttcttctttcatccatccatcttgtatccttttgcttagcctttttgtttggttttcttcctctcgttaaccaccacattcgctctatcttaatacaaaccacccacactcgttctatagcatctgtcttctttcgttcacctcctcac

SEQ ID NO: 19 - DNA, 593 bp, synthetic construct
  source 1..593: mol_type = other DNA
acttaacgttactgaaatcatcaaacagcttgacgaatctggatataagatcgttggtgtcgatgtcagctccggagttgagacaaatggtgttcaggatctcgataagatacgttcatttgtccaagcagcaaagagtgccttctagtgatttaatagctccatgtcaacaagaataaaacgcgtttcgggtttacctcttccagatacagctcatctgcaatgcattaatgcattggacctcgcaaccctagtacgcccttcaggctccggcgaagcagaagaatagcttagcagagtctattttcattttcgggagacgagatcaagcagatcaacggtcgtcaagagacctacgagactgaggaatccgctcttggctccacgcgactatatatttgtctctaattgtactttgacatgctcctcttctttactctgatagcttgactatgaaaattccgtcaccagcccctgggttcgcaaagataattgcactgtttcttccttgaactctcaagcctacaggacacacattcatcgtaggtataaacctcgaaaatcattcctactaagatgggtatacaatagta

SEQ ID NO: 20 - DNA, 522 bp, synthetic construct
  source 1..522: mol_type = other DNA
ataaatgaagaattttgtgaaacgagcgatctacacttgttccttaaggaaaagtaaaactgagatgaatgtaatgtaccatgacttcaaattaataaatcaagatttgcctgcctgtcttttaaacatatatatacacagaaatctaattttaaaccgttactgcagctacaggccctagactgtgacaatggctacgtttcatttagccacacacacacacatcgcagacatcgctgcgatcactgtagatataactcagataaacattcgcttcaggaataaagcgcatggaatccctcagaatgaagaagtacaagaaagcccgccccattggttgtgccattacagagcactaccatatatcacgcgaggcgcgatagggccatctatttggactagtttcactgcagcctaccctggaagtggtctagggtagggatttgctccttaagttgactgctaccatggggtcttgcttcagatgttatggctgaattggactgacttgtgcgctgcaat

SEQ ID NO: 21 - DNA, 37 bp, synthetic construct
  source 1..37: mol_type = other DNA
ctcatcaatcatcacaacatgaagatcccctgcttcg

SEQ ID NO: 22 - DNA, 40 bp, synthetic construct
  source 1..40: mol_type = other DNA
tcagtaacgttaagtggatccttaggggatgatcagctcg

SEQ ID NO: 23 - DNA, 40 bp, synthetic construct
  source 1..40: mol_type = other DNA
cgagctgatcatcccctaaggatccacttaacgttactga

SEQ ID NO: 24 - DNA, 37 bp, synthetic construct
  source 1..37: mol_type = other DNA
cgaagcaggggatcttcatgttgtgatgattgatgag

SEQ ID NO: 25 - DNA, 25 bp, synthetic construct
  source 1..25: mol_type = other DNA
ttacactctgggaggatccaggtac

SEQ ID NO: 26 - DNA, 21 bp, synthetic construct
  source 1..21: mol_type = other DNA
gtcgtgccagtcgactctaga

SEQ ID NO: 27 - DNA, 40 bp, synthetic construct
  source 1..40: mol_type = other DNA
acgaagcaggggatcttcatggtgatgtctgctcaagcgg

SEQ ID NO: 28 - DNA, 21 bp, synthetic construct
  source 1..21: mol_type = other DNA
ttgatcgagacctaatacagc

SEQ ID NO: 29 - DNA, 38 bp, synthetic construct
  source 1..38: mol_type = other DNA
gcatcattacacctcagcaatgaagatcccctgcttcg

SEQ ID NO: 30 - DNA, 25 bp, synthetic construct
  source 1..25: mol_type = other DNA
ggattgcctgaacattgacattcgg

SEQ ID NO: 31 - DNA, 26 bp, synthetic construct
  source 1..26: mol_type = other DNA
tgctgaggtgtaatgatgctggggat

SEQ ID NO: 32 - DNA, 38 bp, synthetic construct
  source 1..38: mol_type = other DNA
cctcttaaattgaccatgaatgaagatcccctgcttcg

SEQ ID NO: 33 - DNA, 25 bp, synthetic construct
  source 1..25: mol_type = other DNA
ctaccaacagtctcgcggtgaatag

SEQ ID NO: 34 - DNA, 25 bp, synthetic construct
  source 1..25: mol_type = other DNA
ggtcaatttaagaggacgatcttcg

SEQ ID NO: 35 - DNA, 43 bp, synthetic construct
  source 1..43: mol_type = other DNA
accgacttctcatccatcttcaaaatgaagatcccctgcttcg

SEQ ID NO: 36 - DNA, 24 bp, synthetic construct
  source 1..24: mol_type = other DNA
gtacagtggccatgaaatccaatc

SEQ ID NO: 37 - DNA, 24 bp, synthetic construct
  source 1..24: mol_type = other DNA
tttgaagatggatgagaagtcggt

SEQ ID NO: 38 - DNA, 41 bp, synthetic construct
  source 1..41: mol_type = other DNA
cctcgcatagagagcttccatcatgaagatcccctgcttcg

SEQ ID NO: 39 - DNA, 18 bp, synthetic construct
  source 1..18: mol_type = other DNA
tggcaccggtccgcggga

SEQ ID NO: 40 - DNA, 22 bp, synthetic construct
  source 1..22: mol_type = other DNA
gatggaagctctctatgcgagg

SEQ ID NO: 41 - DNA, 46 bp, synthetic construct
  source 1..46: mol_type = other DNA
cttttttagactcttgttggattcaaaatgaagatcccctgcttcg

SEQ ID NO: 42 - DNA, 18 bp, synthetic construct
  source 1..18: mol_type = other DNA
caaccaaggaccgcgatg

SEQ ID NO: 43 - DNA, 26 bp, synthetic construct
  source 1..26: mol_type = other DNA
ttgaatccaacaagagtctaaaaaag

SEQ ID NO: 44 - DNA, 46 bp, synthetic construct
  source 1..46: mol_type = other DNA
gcccgcaaggctgctagcaactaaggatccacttaacgttactgaa

SEQ ID NO: 45 - DNA, 21 bp, synthetic construct
  source 1..21: mol_type = other DNA
attacctctaaacaagtgtac

SEQ ID NO: 46 - DNA, 43 bp, synthetic construct
  source 1..43: mol_type = other DNA
cgcaggccacgcttcactgtcgaaatgaagatcccctgcttcg

SEQ ID NO: 47 - DNA, 27 bp, synthetic construct
  source 1..27: mol_type = other DNA
ctttaacgttgcagatacagggatgcg

SEQ ID NO: 48 - DNA, 24 bp, synthetic construct
  source 1..24: mol_type = other DNA
ttcgacagtgaagcgtggcctgcg

SEQ ID NO: 49 - DNA, 43 bp, synthetic construct
  source 1..43: mol_type = other DNA
gtcttctttcgttcacctcctcacatgaagatcccctgcttcg

SEQ ID NO: 50 - DNA, 24 bp, synthetic construct
  source 1..24: mol_type = other DNA
ctgctctctctctgctctctttct

SEQ ID NO: 51 - DNA, 24 bp, synthetic construct
  source 1..24: mol_type = other DNA
gtgaggaggtgaacgaaagaagac

SEQ ID NO: 52 - DNA, 21 bp, synthetic construct
  source 1..21: mol_type = other DNA
ttcgggatcgcaagcgtaaag

SEQ ID NO: 53 - DNA, 22 bp, synthetic construct
  source 1..22: mol_type = other DNA
caattatctttgcgaacccagg

SEQ ID NO: 54 - DNA, 26 bp, synthetic construct
  source 1..26: mol_type = other DNA
ttacactctgggaggatccaggtact

SEQ ID NO: 55 - DNA, 40 bp, synthetic construct
  source 1..40: mol_type = other DNA
ctcatcaatcatcacaacatgctgcaccccatcgacacca

SEQ ID NO: 56 - DNA, 40 bp, synthetic construct
  source 1..40: mol_type = other DNA
tcagtaacgttaagtggatccttaggacaggctacggtcg

SEQ ID NO: 57 - DNA, 40 bp, synthetic construct
  source 1..40: mol_type = other DNA
cgaccgtagcctgtcctaaggatccacttaacgttactga

SEQ ID NO: 58 - DNA, 40 bp, synthetic construct
  source 1..40: mol_type = other DNA
tggtgtcgatggggtgcagcatgttgtgatgattgatgag

SEQ ID NO: 59 - DNA, 43 bp, synthetic construct
  source 1..43: mol_type = other DNA
ccgcttgagcagacatcaccatgctgcaccccatcgacaccat

SEQ ID NO: 60 - DNA, 42 bp, synthetic construct
  source 1..42: mol_type = other DNA
tggtgtcgatggggtgcagcatggtgatgtctgctcaagcgg

SEQ ID NO: 61 - DNA, 41 bp, synthetic construct
  source 1..41: mol_type = other DNA
gcatcattacacctcagcaatgctgcaccccatcgacacca

SEQ ID NO: 62 - DNA, 41 bp, synthetic construct
  source 1..41: mol_type = other DNA
cctcttaaattgaccatgaatgctgcaccccatcgacacca

SEQ ID NO: 63 - DNA, 46 bp, synthetic construct
  source 1..46: mol_type = other DNA
accgacttctcatccatcttcaaaatgctgcaccccatcgacacca

SEQ ID NO: 64 - DNA, 44 bp, synthetic construct
  source 1..44: mol_type = other DNA
cctcgcatagagagcttccatcatgctgcaccccatcgacacca

SEQ ID NO: 65 - DNA, 49 bp, synthetic construct
  source 1..49: mol_type = other DNA
cttttttagactcttgttggattcaaaatgctgcaccccatcgacacca

SEQ ID NO: 66 - DNA, 46 bp, synthetic construct
  source 1..46: mol_type = other DNA
cgcaggccacgcttcactgtcgaaatgctgcaccccatcgacacca

SEQ ID NO: 67 - DNA, 46 bp, synthetic construct
  source 1..46: mol_type = other DNA
gtcttctttcgttcacctcctcacatgctgcaccccatcgacacca

SEQ ID NO: 68 - DNA, 20 bp, synthetic construct
  source 1..20: mol_type = other DNA
gggcaattgattacgggatc

SEQ ID NO: 69 - DNA, 20 bp, synthetic construct
  source 1..20: mol_type = other DNA
atggggtgacgatgagccgc

SEQ ID NO: 70 - DNA, 49 bp, synthetic construct
  source 1..49: mol_type = other DNA
aacaactcatcaatcatcacaacatgatctccacccgccttgcgcgcat

SEQ ID NO: 71 - DNA, 46 bp, synthetic construct
  source 1..46: mol_type = other DNA
ttcagtaacgttaagtggatccttagttgctagcagccttgcgggc

SEQ ID NO: 72 - DNA, 49 bp, synthetic construct
  source 1..49: mol_type = other DNA
atgcgcgcaaggcgggtggagatcatgttgtgatgattgatgagttgtt

SEQ ID NO: 73 - DNA, 46 bp, synthetic construct
  source 1..46: mol_type = other DNA
ccgcttgagcagacatcaccatgatctccacccgccttgcgcgcat

SEQ ID NO: 74 - DNA, 46 bp, synthetic construct
  source 1..46: mol_type = other DNA
atgcgcgcaaggcgggtggagatcatggtgatgtctgctcaagcgg

SEQ ID NO: 75 - DNA, 47 bp, synthetic construct
  source 1..47: mol_type = other DNA
cagcatcattacacctcagcaatgatctccacccgccttgcgcgcat

SEQ ID NO: 76 - DNA, 45 bp, synthetic construct
  source 1..45: mol_type = other DNA
cctcttaaattgaccatgaatgatctccacccgccttgcgcgcat

SEQ ID NO: 77 - DNA, 50 bp, synthetic construct
  source 1..50: mol_type = other DNA
accgacttctcatccatcttcaaaatgatctccacccgccttgcgcgcat

SEQ ID NO: 78 - DNA, 48 bp, synthetic construct
  source 1..48: mol_type = other DNA
cctcgcatagagagcttccatcatgatctccacccgccttgcgcgcat

SEQ ID NO: 79 - DNA, 53 bp, synthetic construct
  source 1..53: mol_type = other DNA
cttttttagactcttgttggattcaaaatgatctccacccgccttgcgcgcat

SEQ ID NO: 80 - DNA, 50 bp, synthetic construct
  source 1..50: mol_type = other DNA
cgcaggccacgcttcactgtcgaaatgatctccacccgccttgcgcgcat

SEQ ID NO: 81 - DNA, 50 bp, synthetic construct
  source 1..50: mol_type = other DNA
gtcttctttcgttcacctcctcacatgatctccacccgccttgcgcgcat

SEQ ID NO: 82 - DNA, 40 bp, synthetic construct
  source 1..40: mol_type = other DNA
ccgcttgagcagacatcaccatgaagatcccctgcttcgt

SEQ ID NO: 83 - DNA, 19 bp, synthetic construct
  source 1..19: mol_type = other DNA
tcatggtcaatttaagagg

SEQ ID NO: 84 - DNA, 20 bp, synthetic construct
  source 1..20: mol_type = other DNA
cccggagttaggtagataga

SEQ ID NO: 85 - DNA, 21 bp, synthetic construct
  source 1..21: mol_type = other DNA
gcatcaaatcgtcgtaccgca

SEQ ID NO: 86 - DNA, 42 bp, synthetic construct
  source 1..42: mol_type = other DNA
gcggtacgacgatttgatgcttacactctgggaggatccagg

SEQ ID NO: 87 - DNA, 20 bp, synthetic construct
  source 1..20: mol_type = other DNA
gttgtgatgattgatgagtt

SEQ ID NO: 88 - DNA, 43 bp, synthetic construct
  source 1..43: mol_type = other DNA
tctgagagaggcagccatgttgtgatgattgatgagttgttgg

SEQ ID NO: 89 - DNA, 40 bp, synthetic construct
  source 1..40: mol_type = other DNA
gcaaggcgggtggagatcatgttgtgatgattgatgagtt

SEQ ID NO: 90 - DNA, 40 bp, synthetic construct
  source 1..40: mol_type = other DNA
ctgaaccggacagacgacatgttgtgatgattgatgagtt

SEQ ID NO: 91 - DNA, 19 bp, synthetic construct
  source 1..19: mol_type = other DNA
atggctgcctctctcagac

SEQ ID NO: 92 - DNA, 20 bp, synthetic construct
  source 1..20: mol_type = other DNA
gtagcagcgcaagccattga

SEQ ID NO: 93 - DNA, 19 bp, synthetic construct
  source 1..19: mol_type = other DNA
atgatctccacccgccttg

SEQ ID NO: 94 - DNA, 21 bp, synthetic construct
  source 1..21: mol_type = other DNA
ataggggaatcagcaacggtg

SEQ ID NO: 95 - DNA, 20 bp, synthetic construct
  source 1..20: mol_type = other DNA
atgtcgtctgtccggttcag

SEQ ID NO: 96 - DNA, 20 bp, synthetic construct
  source 1..20: mol_type = other DNA
ggtgcgggattgagtaaggt

SEQ ID NO: 97 - DNA, 40 bp, synthetic construct
  source 1..40: mol_type = other DNA
ctcatcaatcatcacaacatggcctccacccccttcaagt

SEQ ID NO: 98 - DNA, 36 bp, synthetic construct
  source 1..36: mol_type = other DNA
aatggcttgcgctgctacatggcctccacccccttc

SEQ ID NO: 99 - DNA, 36 bp, synthetic construct
  source 1..36: mol_type = other DNA
accgttgctgattcccctatggcctccacccccttc

SEQ ID NO: 100 - DNA, 40 bp, synthetic construct
  source 1..40: mol_type = other DNA
accttactcaatcccgcaccatggcctccacccccttcaa

SEQ ID NO: 101 - DNA, 41 bp, synthetic construct
  source 1..41: mol_type = other DNA
attctatctacctaactccgggttacaggtgggcctccagg

SEQ ID NO: 102 - DNA, 23 bp, synthetic construct
  source 1..23: mol_type = other DNA
gggtttctagaagtcacatcagc

SEQ ID NO: 103 - DNA, 20 bp, synthetic construct
  source 1..20: mol_type = other DNA
atcaccgaccctacgctgtg

SEQ ID NO: 104 - DNA, 22 bp, synthetic construct
  source 1..22: mol_type = other DNA
atataccactccacactaaccg

SEQ ID NO: 105 - DNA, 21 bp, synthetic construct
  source 1..21: mol_type = other DNA
gccatagagttgctcttgatc

SEQ ID NO: 106 - DNA, 21 bp, synthetic construct
  source 1..21: mol_type = other DNA
gcgataaatgttgaacgaggc

SEQ ID NO: 107 - DNA, 44 bp, synthetic construct
  source 1..44: mol_type = other DNA
agtctgagagaggcagccatggtcaatttaataggacaattttc

SEQ ID NO: 108 - DNA, 41 bp, synthetic construct
  source 1..41: mol_type = other DNA
aggcgggtggagatcatggtcaatttaataggacaattttc

SEQ ID NO: 109 - DNA, 20 bp, synthetic construct
  source 1..20: mol_type = other DNA
atggctgcctctctcagact

SEQ ID NO: 110 - DNA, 20 bp, synthetic construct
  source 1..20: mol_type = other DNA
gtagcagcgcaagccattga

SEQ ID NO: 111 - DNA, 19 bp, synthetic construct
  source 1..19: mol_type = other DNA
atgatctccacccgccttg

SEQ ID NO: 112 - DNA, 21 bp, synthetic construct
  source 1..21: mol_type = other DNA
ataggggaatcagcaacggtg

SEQ ID NO: 113 - DNA, 41 bp, synthetic construct
  source 1..41: mol_type = other DNA
ttcaatggcttgcgctgctacatgctgcaccccatcgacac

SEQ ID NO: 114 - DNA, 41 bp, synthetic construct
  source 1..41: mol_type = other DNA
gccaccgttgctgattcccctatgctgcaccccatcgacac

SEQ ID NO: 115 - DNA, 40 bp, synthetic construct
  source 1..40: mol_type = other DNA
caatggcttgcgctgctacatgaagatcccctgcttcgtc

SEQ ID NO: 116 - DNA, 40 bp, synthetic construct
  source 1..40: mol_type = other DNA
aattgtcctattaaattgaccatgatctccacccgccttg

SEQ ID NO: 117 - DNA, 20 bp, synthetic construct
  source 1..20: mol_type = other DNA
ttaggggatgatcagctcgc

SEQ ID NO: 118 - DNA, 40 bp, synthetic construct
  source 1..40: mol_type = other DNA
gcgaccgtagcctgtcctaaggatccacttaacgttactg

SEQ ID NO: 119 - DNA, 40 bp, synthetic construct
  source 1..40: mol_type = other DNA
gcgagctgatcatcccctaaggatccacttaacgttactg

SEQ ID NO: 120 - DNA, 22 bp, synthetic construct
  source 1..22: mol_type = other DNA
aagaaggttacctctaaacaag

SEQ ID NO: 121 - DNA, 46 bp, synthetic construct
  source 1..46: mol_type = other DNA
cttgtttagaggtaaccttctttaagggagatggtgattgaactag

SEQ ID NO: 122 - DNA, 21 bp, synthetic construct
  source 1..21: mol_type = other DNA
gcatcaaatcgtcgtaccgca

SEQ ID NO: 123 - DNA, 41 bp, synthetic construct
  source 1..41: mol_type = other DNA
tgcggtacgacgatttgatgcatgggaagcgatatggaaac

SEQ ID NO: 124 - DNA, 23 bp, synthetic construct
  source 1..23: mol_type = other DNA
cattgcagggaagtatatgcttc

SEQ ID NO: 125 - DNA, 21 bp, synthetic construct
  source 1..21: mol_type = other DNA
tgtggttcctaccaaggtggc

SEQ ID NO: 126 - DNA, 22 bp, synthetic construct
  source 1..22: mol_type = other DNA
cgactatagctggattgatcac

SEQ ID NO: 127 - DNA, 20 bp, synthetic construct
  source 1..20: mol_type = other DNA
ttcgacagtgaagcgtggcc

SEQ ID NO: 128 - DNA, 40 bp, synthetic construct
  source 1..40: mol_type = other DNA
ggccacgcttcactgtcgaaatgtcgtctgtccggttcag

SEQ ID NO: 129 - DNA, 43 bp, synthetic construct
  source 1..43: mol_type = other DNA
gacgaagcaggggatcttcatggtgcgggattgaggaaggttc

SEQ ID NO: 130 - DNA, 21 bp, synthetic construct
  source 1..21: mol_type = other DNA
atgaagatcccctgcttcgtc

SEQ ID NO: 131 - DNA, 21 bp, synthetic construct
  source 1..21: mol_type = other DNA
ttaggggatgatcagctcgcc

SEQ ID NO: 132 - DNA, 49 bp, synthetic construct
  source 1..49: mol_type = other DNA
ggcgagctgatcatcccctaaggatccacttaacgttactgaaatcatc

SEQ ID NO: 133 - DNA, 24 bp, synthetic construct
  source 1..24: mol_type = other DNA
gaatcagagctccatcatgtcttg

SEQ ID NO: 134 - DNA, 40 bp, synthetic construct
  source 1..40: mol_type = other DNA
gtgtcgatggggtgcagcatggtgcgggattgaggaaggt

SEQ ID NO: 135 - DNA, 20 bp, synthetic construct
  source 1..20: mol_type = other DNA
atgctgcaccccatcgacac

SEQ ID NO: 136 - DNA, 20 bp, synthetic construct
  source 1..20: mol_type = other DNA
ttaggacaggctacggtcgc

SEQ ID NO: 137 - DNA, 1188 bp, synthetic construct
  source 1..1188: mol_type = other DNA
gcgataaatgttgaacgaggcaaattctgtttgttattgcaaacggtcatttcttttcgttccacgcgggcttataaggtggatcgctacatacgaacggaggctttcaatgtggttcctaccaaggtggctccatatccagcataccagcctcggattccaggtcttatagctgccacatcatggtttcggcgcttaagctgggcgcgagttttagccgctaccagcggaagcaatagattgtcagttggcggccacggtaaagcagaattcttaaacacaagatatgctcacattcgaaagggtaggtgatggagatttcaacagccccagcacaagcacccgcaaccaatgcaggaatacctttcgtctatacatatattaagaaaagacattgtcagtatcatggcccaagcgcgaccaagaaggaacacatacacgcttgccacgagctttttgggtaaggggtgcctttggtaatggaacacttgtctggactttagagtccatgacggcgatgtgctgagtccaaacaaagcttttcttcacagagatagggctgtagactttatttccagtttgccttccctgtgttcagtatcgggtcttatattgtattatctcaatgcttatgactctgagtggaatgcattggatatcagtttgtcacggagtcggcacccgatggctatcgcaatcgtccctggtgggtcttgaaatcgtatgccacacttgctccggatgaaacacattccggagcgcgcatcgatattgctacacagtatagacccaatggtctgcagatgccctaaatggtagttctcactggcctgcattaagttctggttgcagatcattgtcggcctaacatcagtgtaggttacggtgtgagatttacttgcatagaagattccagaccacaaggttctagatcctttgacggcggactcccctcgaggtgccgggcgccgacgtgtgcgttgctccgggatttgtaggacgcagctcggatacctagccgttatgggaatcggaggttgtagcagcgtaaacacatggatagttaaataatcggatgtacacccactgttggaaatgacgggggcctacaacacgagattatctgatccaatttctgttcgttggcattctatcattcgcagcgaaaattgtcctattaaattgacc

SEQ ID NO: 138 - DNA, 1255 bp, synthetic construct
  source 1..1255: mol_type = other DNA
atgggaagcgatatggaaacatttcatgtcacgggcacaaattctaggtcatatcgtacctggatggtgaaaccaccagcggtttagcagatagaagatagactccttctgctctgcgttgcgtcttgaatttagttcgttcactggcttaagaacttagaatgcaatacagtctctcttatttcttattaaaatcacgtattcccacattcggcgactggaggatacgaaagcagtgttggtggtgctccccgtaatggatatgattttgctgactggactattctatgaccattccctccaacggagatcctttctcgacactttagatgttgacgctgtctggaggaactacttttgcgctgcaaagactatgagcagtggagctgcatcttttcgattagatatccattctgcatagctacaaggcaaggtttcacaaaaatagttcactgtacgtcaatgccagcggaacagccgcttaaacaagtcgatacattaaatactgcctataagcaaccgcctgtataaggaatcctgcgatattagcaactaacattctcgtctaaatttatttcctatctaaatcagcaattaatctgaatacaaagttattacttaaaataccctctctcctatacaaagttacttataggaaataacttaattagaaaatataggtttaactggctaaaagtctaccttgaaacattatattgtaacattgttagacaattatgtgaccactcaagtagaaatatatatcttagagagattacctccttagtagaatatatatttgtatagacctgactgtaagcaatttcttattataagtaactttttttgatgagctgaattcgttgcttatagccagcttttgctgtgattcgtaaaaggtgccaattctccgtaatgtgtcccgcatccgatgaactgttgacgacccacaccataaactgcatcatgatctacattttcctcattggtatctattgggtaggcatattgaaagccttttctgcccatctttgcatatttatcccccaccttgcgatggccgccgtgatcaatccagctatagtcgaagcaaccacacctgtaagaactgtgagcatgtacattgagaggtgggaagaaaagtaccatacatagcgtgaacgtccatccaactccgagggcgtttatcacgagatcaacgactgcactacttcctgcagaaaaggagtattgaagcatatacttccctgcaatg

SEQ ID NO: 139 - DNA, 654 bp, synthetic construct
  source 1..654: mol_type = other DNA
atggcctccacccccttcaagtttcagctcaagggcaccatcaacggcaagtccttcaccgtcgagggcgagggcgagggcaactcccacgagggctcccacaagggcaagtacgtctgcacctccggcaagctccccatgtcctgggccgccctcggcacgtccttcggctacggcatgaagtactacaccaagtacccctccggcctcaagaactggttccacgaggtcatgcccgagggcttcacctacgaccgccacattcagtacaagggcgacggctccatccacgccaagcatcagcacttcatgaagaacggcacctaccacaacatcgtcgagttcaccggccaagacttcaaggagaactcccccgtcctcaccggcgacatgaacgtctccctccccaacgaggttcagcacatcccccgcgacgacggcgtcgagtgccccgtcaccctcctctaccccctcctctccgacaagtccaagtgcgtcgaggcccatcagaacaccatctgcaagcccctccacaatcagcccgcccccgacgtcccctaccactggattcgcaagcagtacacgcagtccaaggacgacaccgaggagcgcgaccacatctgtcagtccgagaccctggaggcccacctgtaa